European Patent Application EP 4 112 058 A1, published January 4, 2023. Title: Tetracycline derivative induced mitohormesis mediates disease tolerance against viral infections. Applicant: Ecole Polytechnique Federale de Lausanne (EPFL). The sequence listing filed with the application follows.

SEQUENCE LISTING (34 sequences)

SEQ ID NO: 1 - DNA, 20 bp, Artificial Sequence
  Asns forward primer
ttgacccgctgtttggaatg

SEQ ID NO: 2 - DNA, 23 bp, Artificial Sequence
  Asns reverse primer
cgccttgtggttgtagatttcac

SEQ ID NO: 3 - DNA, 20 bp, Artificial Sequence
  Chop/Ddit3 forward primer
cggaacctgaggagagagtg

SEQ ID NO: 4 - DNA, 20 bp, Artificial Sequence
  Chop/Ddit3 reverse primer
cgtttcctggggatgagata

SEQ ID NO: 5 - DNA, 19 bp, Artificial Sequence
  Lonp1 forward primer
atgaccgtcccggatgtgt

SEQ ID NO: 6 - DNA, 22 bp, Artificial Sequence
  Lonp1 reverse primer
cctccacgatcttgataaagcg

SEQ ID NO: 7 - DNA, 20 bp, Artificial Sequence
  Hspa9 forward primer
aatgagagcgctccttgctg

SEQ ID NO: 8 - DNA, 20 bp, Artificial Sequence
  Hspa9 reverse primer
ctgttccccagtgccagaac

SEQ ID NO: 9 - DNA, 22 bp, Artificial Sequence
  Hspe1 forward primer
ctgacaggttcaatctctccac

SEQ ID NO: 10 - DNA, 20 bp, Artificial Sequence
  Hspe1 reverse primer
aggtggcattatgcttccag

SEQ ID NO: 11 - DNA, 21 bp, Artificial Sequence
  Cxcl10 forward primer
ccacgtgttgagatcattgcc

SEQ ID NO: 12 - DNA, 20 bp, Artificial Sequence
  Cxcl10 reverse primer
gaggctctctgctgtccatc

SEQ ID NO: 13 - DNA, 27 bp, Artificial Sequence
  Ifi44 forward primer
ctgattacaaaagaagacatgacagac

SEQ ID NO: 14 - DNA, 20 bp, Artificial Sequence
  Ifi44 reverse primer
aggcaaaaccaaagactcca

SEQ ID NO: 15 - DNA, 20 bp, Artificial Sequence
  Ddx58 forward primer
atgtgcccctactggttgtg

SEQ ID NO: 16 - DNA, 20 bp, Artificial Sequence
  Ddx58 reverse primer
ccccagaaatgctcgcaatg

SEQ ID NO: 17 - DNA, 19 bp, Artificial Sequence
  Ifit3 forward primer
ttcccagcagcacagaaac

SEQ ID NO: 18 - DNA, 20 bp, Artificial Sequence
  Ifit3 reverse primer
aaattccaggtgaaatggca

SEQ ID NO: 19 - DNA, 20 bp, Artificial Sequence
  Irf7 forward primer
caattcaggggatccagttg

SEQ ID NO: 20 - DNA, 20 bp, Artificial Sequence
  Irf7 reverse primer
agcattgctgaggctcactt

SEQ ID NO: 21 - DNA, 21 bp, Artificial Sequence
  36B4 forward primer
agattcgggatatgctgttgg

SEQ ID NO: 22 - DNA, 21 bp, Artificial Sequence
  36B4 reverse primer
aaagcctggaagaaggaggtc

SEQ ID NO: 23 - DNA, 17 bp, Artificial Sequence
  Actb forward primer
gagaccttcaacacccc

SEQ ID NO: 24 - DNA, 20 bp, Artificial Sequence
  Actb reverse primer
gtggtggtgaagctgtagcc

SEQ ID NO: 25 - DNA, 21 bp, Artificial Sequence
  HSPA9 forward primer
tggtgagcgacttgttggaat

SEQ ID NO: 26 - DNA, 21 bp, Artificial Sequence
  HSPA9 reverse primer
attggaggcacggacaatttt

SEQ ID NO: 27 - DNA, 19 bp, Artificial Sequence
  LONP1 forward primer
cccgcgctttatcaagatt

SEQ ID NO: 28 - DNA, 20 bp, Artificial Sequence
  LONP1 reverse primer
agaaagacgccgacataagg

SEQ ID NO: 29 - DNA, 20 bp, Artificial Sequence
  ASNS forward primer
atcactgtcgggatgtaccc

SEQ ID NO: 30 - DNA, 20 bp, Artificial Sequence
  ASNS reverse primer
tgataaaaggcagccaatcc

SEQ ID NO: 31 - DNA, 22 bp, Artificial Sequence
  CHOP forward primer
acagtgtcccgaaggagaaagg

SEQ ID NO: 32 - DNA, 22 bp, Artificial Sequence
  CHOP reverse primer
gccaaaatcagagctggaacct

SEQ ID NO: 33 - DNA, 20 bp, Artificial Sequence
  ACTB forward primer
tcgtgcgtgacattaaggag

SEQ ID NO: 34 - DNA, 20 bp, Artificial Sequence
  ACTB reverse primer
gtcaggcagctcgtagctct